European Patent Application EP 4 556 909 A1, published May 21, 2025. Title: AN IN VITRO METHOD FOR DETECTING CANCER. Applicant: Inmunotek SL. The sequence listing filed with the application follows.

SEQUENCE LISTING (20 sequences)

SEQ ID NO: 1 - DNA, 21 bp, synthetic construct
  source 1..21: mol_type = other DNA
ggtacatcctcgacggcatct

SEQ ID NO: 2 - DNA, 21 bp, synthetic construct
  source 1..21: mol_type = other DNA
gtgcctctttgctgctttcac

SEQ ID NO: 3 - DNA, 21 bp, synthetic construct
  source 1..21: mol_type = other DNA
tttttgctgtgagtcccggag

SEQ ID NO: 4 - DNA, 22 bp, synthetic construct
  source 1..22: mol_type = other DNA
ttcgacacatgggataacgagg

SEQ ID NO: 5 - DNA, 19 bp, synthetic construct
  source 1..19: mol_type = other DNA
gtgatgccccaagctgaga

SEQ ID NO: 6 - DNA, 20 bp, synthetic construct
  source 1..20: mol_type = other DNA
cacggccttgctcttgtttt

SEQ ID NO: 7 - DNA, 30 bp, synthetic construct
  source 1..30: mol_type = other DNA
aagatgaggatatttgctgtctttatattc

SEQ ID NO: 8 - DNA, 21 bp, synthetic construct
  source 1..21: mol_type = other DNA
gtccttgggaaccgtgacagt

SEQ ID NO: 9 - DNA, 20 bp, synthetic construct
  source 1..20: mol_type = other DNA
agaagtgggctttgctctgc

SEQ ID NO: 10 - DNA, 23 bp, synthetic construct
  source 1..23: mol_type = other DNA
tggcaagaccttacggacatctc

SEQ ID NO: 11 - DNA, 21 bp, synthetic construct
  source 1..21: mol_type = other DNA
ccctggttgttgtagcagctt

SEQ ID NO: 12 - DNA, 19 bp, synthetic construct
  source 1..19: mol_type = other DNA
caacccctggtttgtgcaa

SEQ ID NO: 13 - DNA, 22 bp, synthetic construct
  source 1..22: mol_type = other DNA
cctcagcatctctgtcggaaga

SEQ ID NO: 14 - DNA, 22 bp, synthetic construct
  source 1..22: mol_type = other DNA
gcatcgtactggtccaggaact

SEQ ID NO: 15 - DNA, 19 bp, synthetic construct
  source 1..19: mol_type = other DNA
ctgccgggaaaagcaatct

SEQ ID NO: 16 - DNA, 24 bp, synthetic construct
  source 1..24: mol_type = other DNA
aaattcaacagcattgtccaagtc

SEQ ID NO: 17 - DNA, 20 bp, synthetic construct
  source 1..20: mol_type = other DNA
agggcagttcttgcaaccat

SEQ ID NO: 18 - DNA, 25 bp, synthetic construct
  source 1..25: mol_type = other DNA
gcgtaatatcgaaaggttttgatga

SEQ ID NO: 19 - DNA, 18 bp, synthetic construct
  source 1..18: mol_type = other DNA
gccgtgtggcaatccaat

SEQ ID NO: 20 - DNA, 18 bp, synthetic construct
  source 1..18: mol_type = other DNA
gccgtgtggcaatccaat